European Patent Application EP 4 644 540 A1, published November 5, 2025. Title: ENZYME, STRAIN FOR PRODUCING SALIDROSIDE, AND PRODUCTION METHOD. Applicant: Bloomage Biotechnology Corporation Limited. The sequence listing filed with the application follows.

SEQUENCE LISTING (28 sequences)

SEQ ID NO: 1 - DNA, 1539 bp, Synthetic construct
  source 1..1539: mol_type = other DNA
atgggttctttgccaaccaacaaccttgaatctatttccttatgctctcaaaacccattagacccagacgaattcagaagacaaggtcacatgatcattgatttcttggctgattactacaagaacgttgaaaagtacccagtcagatcccaagtcgaaccaggctacttaaagaagagattgccagagtctgctccatacaacccagaatccatcgaaaccatcttggaagatgtcacaaacgatatcatcccaggtttgacccactggcaatctccaaattactttgcttacttcccatcttctggttctatcgccggttttttaggtgaaatgttgtctaccggtttcaatgttgtcggtttcaactggatgtctagtccagctgccactgaattggaatctattgttatgaactggttgggtcaaatgttgactttgccaaaatctttcttattctcttctgatggttcctccggtggtggtggtgtcttgcaaggtactacttgtgaagctatcttgtgtactttgaccgctgctagagacaagatgctgaataaaattggtagagaaaacattaacaagttggttgtctacgcttccgatcaaactcattgtgctttgcaaaaggccgctcaaattgctggtattaaccctaaaaatgttagagctatcaagacctctaaggctactaacttcggtttgagcccgaactctttgcaatccgccattctagccgatattgaatccggattggttcctttgttcttgtgcgctactgtcggtaccacttcaagcactgctgtcgatccaatcggtccattgtgtgctgttgccaagttgtacggtatctgggttcacatagatgctgcttatgccggttccgcttgtatctgtccagaattccgtcactttattgacggtgttgaagacgctgactctttctccttgaacgctcacaagtggttcttcaccaccttggactgttgttgtttgtgggtcaaggattccgactccttggtcaaagctttatctacctctccagaatttttgaagaacaaggctaccgaatccaagcaagttattgactacaaggactggcaaatcgctttgtcacgtagattcagatccatgaagctatggttagttttgagatcttacggtgttgctaacttgagaaccttcttgcgttctcatgtcaagatggctaagcatttccaaggtttgattggtatggacaacagatacgaaatcgttgtcccaagaactttcgctatggtttgtttcagattaaagccaactgccatcttcaagcaaaagattgttgacaacgactacattgaagaccaaacgaacgaagtcaacgtcaaattgttggaatctgttaacgcttctggtaagatctatatgactcacgctgtcgttggtggtgtttacatgatcagatttgccgtaggtgccaccctcactgaagaaagacacgttactggtgcttggaaggttgttcaagaacacactgatgcaatcttgggtgcttga

SEQ ID NO: 2 - DNA, 1539 bp, Synthetic construct
  source 1..1539: mol_type = other DNA
atgggaagccttccgactaataaccttgagagcatctcactgtgttcgcaaaatccacttgatccagatgaattcagaaggcaaggtcacatgattattgatttccttgctgattactacaaaaatgttgagaagtatccagttagaagccaagtcgagcccggttatttgaagaaacggttacccgaatctgctccatacaatcctgaatccattgaaactattcttgaagatgtcacaaatgatatcatacctggtctaactcactggcaaagtccaaattactttgcttactttccttctagtggttccattgctggtttccttggagagatgctaagtaccggatttaatgttgtcggcttcaattggatgtcatctccggctgcaactgagttggagagtattgttatgaattggcttggccagatgcttacgcttcccaaatcatttctcttctcatcagatggaagttcaggaggaggcggtgttttgcaagggactacttgtgaagccattttatgtactctaactgcagcgagagacaaaatgttgaacaaaattggtagagaaaatattaacaagttggttgtttatgcttctgatcaaacccattgtgcacttcaaaaagctgctcagattgctgggattaatccgaagaacgtccgcgctattaaaacgtccaaggctacaaatttcggtctctctccaaattcacttcaatcggcaattcttgcagatatcgaatctgggttagttccgttgttcctctgtgctaccgtcggaacaacttcttcaacagccgtagatcctattggccctctctgcgcggtggcaaaactgtatggtatttgggttcatatcgatgcggcttatgctggaagtgcttgtatctgcccagagttcaggcacttcattgatggtgtggaagatgcagattcatttagtctaaatgcacacaagtggttcttcactacattggattgttgttgtttatgggtgaaagactccgactcccttgttaaagcattatcaacaagtccagaatacttgaagaacaaagcaacggaatcaaaacaagttattgattacaaagactggcaaatagctctcagcagaagattccgatccatgaaactctggttagtccttcgcagctacggggttgctaacttaagaaccttcctcaggagtcatgttaaaatggctaagcattttcaagggctcataggcatggataacaggtttgagattgtggttccaagaacatttgccatggtgtgctttcgccttaaaccaactgcaattttcaagcaaaagatagtcgataatgattacattgaagatcaaacaaatgaggtaaatgtgaaattgcttgaatcagtcaatgcgtccggcaagatatacatgactcatgctgttgtaggaggggtgtacatgattcggtttgccgttggggcaacactgacagaggaaagacatgtgactggggcgtggaaggtagttcaggagcatacagatgccatacttggtgcctag

SEQ ID NO: 3 - DNA, 1701 bp, Synthetic construct
  source 1..1701: mol_type = other DNA
atggaatttggtaccggcaacggctacagcaacgggaacggctacaccaatggaaacggccacaccaacggaaacggcaattacaacggcaatggccacgttaatggtaacggaaaagctaacggagccaaggtggtaaagatgaaaccaatggacagtgagttgctgagagagcaaggtcacataatggttgattttattgctgattattacaaaaaccttcaagactcgcctcaagatttccctgttctgtcccaagttcagcctggttatctccgtgacatgttgcctgattcagcacctgaacgacctgaatcgttaaaagaacttctcgacgatgtttcgaagaagataatgccggggataactcattggcaaagcccgagttactttgcatactatgcatcaagcacgagtgtggctggattcttaggagagatgcttaacgccggcctgagcgtcgtcggttttacctggctcacttctcctgccgctactgagctcgaaatcatcgttcttgattggcttgctaaattgctacaactccccgaccattttctctccacaggaaaaggaaatggaggaggagtaatccaagggacaggatgtgaagcagtgcttgtggtagtattagctgctagagacagaattctgaagaaagttggcaaaacattacttcctcaacttgttgtctatggctctgaccaaacccattctagtttccgaaaagcttgtctgattggtgggatacatgaagaaaacattaggctgctcaaaactgattcttccacaaactatggaatgcctccagaatcacttgaggaagctatttctcatgatctcgctaagggttttatccctttcttcatttgtgccactgttggcacaacgtcttcagcagcggttgatcctttggtcccattggggaacatcgcaaagaaatatgggatatggttgcatgtggatgcagcttatgcagggaatgcatgtatatgtccagaatatcgaaaatttattgacgggattgaaaacgcagactcctttaacatgaatgctcataaatggttatttgctaatcaaacttgttcacctctttgggttaaggatcgatactctctcattgatgctctcaaaacaaatcccgagtatctagaattcaaggtttccaaaaaagatacggtcgtaaattataaagattggcaaatttctctctctcggagattcaggttctttataagtccatttgatgttgtatttgctggtcctattagtctaacaaacttatatgtacacgcatttgatttatacagatcactgaagttatggatggttttacggctctatggttccgagaacttaagaaactttataagagaccatgtcaatctcgctaagcattttgaagattatgtagctcaagatccaagttttgaggttgtcactactcggtacttttcactcgtttgctttcgccttgcgccagttgacggcgatgaagaccaatgtaacgaacgtaaccgtgaactgcttgcggctgttaactccactggcaagatattcatctctcacacggctctatctggaaaattcgttttacgatttgctgttggtgcaccgttaacggaagagaagcatgtcactgaagcatggcagattatacagaaacatgcctccaaatttacacgcaacgaccattattaa

SEQ ID NO: 4 - DNA, 1497 bp, Synthetic construct
  source 1..1497: mol_type = other DNA
atgtctttgatcgaaaagccattgactgccattgaaaccagagaaaagccacacgctgtctgtattccttacccagctcaaggtcacatcaacccaatgatgcaattagccaagttgttgcaccactccggtttccacatcactttcgttcacactgaatacaactacgacagattagtcaaatctcaaggttctgcttgtgttgctggtttgccagacttcagattcgaagctatcccggacggtttgccttctaccaatggtgatgttactcaagacattccattattgtcttcttctacttcaaagacctgtttgaagccattcaaggaattgctcaaaagattgcaagataagtgtaaggaattaccagacgatgttccaccattgtcctgcattgtctccgacgctgctatgtctttcaccatcgatgcttctgaagaattcggtgttccaattgctttgttgtggactgcttccgcctgtggtttcttgggttacacccactacccatacttgatcgacagaggtgtcatcccattgaaggatgaaagccaattgaccaacggttacttggacatgtccatcgatggtattccatgtatggaaggtatcagattgcgtgatttgccatctttcttgagaaccaccgatctagacgacatgatgttctcttacattttgcacgaaattaagcaagtttccagaggttccgctatcatcttgaacactttcgaagctttggaccacgatgttttagattccttgtctaagatttaccaaaacgttattttgccagttggcccattgcatgtttcgttgaacaagatcccaaagcattatccattgcaatctttgtcctctaacttgtggaaggatgacactgactgtatcccatggttaagttccaaggcctctaaatccgttatatacgttaactttggttctatcactactgtctcaccaaaacaaatcgtcgagtttgcttggggtctggccaattccaagcaccctttcttatggattatcagaccagatttggtggctggtgaagcttctattattccacaagatttcatggacgaaactaagggtagaggtttgcttgctggttggtgtgaccaagaattggttttgaaccacccatccattggtggtttcttgactcactgcggctggaactccatcattgaatctatctctgccggtgtcccaaccgtctgttggccattctttgctgaacaacaaaccaactgttggttcgcttgtaagaagtggtgtatcggtatggaaatgcatactgatgtcaagagagacgaagttgacaaattattgagagaattgatggaaggtgacaagggtgaagaattaaagagaaaggctacaaactggaagcgtttggctgaagaagccgtttcttcaactggtctatccaccctaaactttagaactttggtcaaccaagtcttgttgtctaagaccaagcatatccgttga

SEQ ID NO: 5 - DNA, 1908 bp, Synthetic construct
  source 1..1908: mol_type = other DNA
atggcacctgttacaattgaaaagttcgtaaatcaagaagaacgacaccttgtttccaaccgatcagcaacaattccgtttggtgaatacatatttaaaagattgttgtccatcgatacgaaatcagttttcggtgttcctggtgacttcaacttatctctattagaatatctctattcacctagtgttgaatcagctggcctaagatgggtcggcacgtgtaatgaactgaacgccgcttatgcggccgacggatattcccgttactctaataagattggctgtttaataaccacgtatggcgttggtgaattaagcgccttgaacggtatagccggttcgttcgctgaaaatgtcaaagttttgcacattgttggtgtggccaagtccatagattcgcgttcaagtaactttagtgatcggaacctacatcatttggtcccacagctacatgattcaaattttaaagggccaaatcataaagtatatcatgatatggtaaaagatagagtcgcttgctcggtagcctacttggaggatattgaaactgcatgtgaccaagtcgataatgttatccgcgatatttacaagtattctaaacctggttatatttttgttcctgcagattttgcggatatgtctgttacatgtgataatttggttaatgttccacgtatatctcaacaagattgtatagtatacccttctgaaaaccaattgtctgacataatcaacaagattactagttggatatattccagtaaaacacctgcgatccttggagacgtactgactgataggtatggtgtgagtaactttttgaacaagcttatctgcaaaactgggatttggaatttttccactgttatgggaaaatctgtaattgatgagtcaaacccaacttatatgggtcaatataatggtaaagaaggtttaaaacaagtctatgaacattttgaactgtgcgacttggtcttgcattttggagtcgacatcaatgaaattaataatgggcattatacttttacttataaaccaaatgctaaaatcattcaatttcatccgaattatattcgccttgtggacactaggcagggcaatgagcaaatgttcaaaggaatcaattttgcccctattttaaaagaactatacaagcgcattgacgtttctaaactttctttgcaatatgattcaaatgtaactcaatatacgaacgaaacaatgcggttagaagatcctaccaatggacaatcaagcattattacacaagttcacttacaaaagacgatgcctaaatttttgaaccctggtgatgttgtcgtttgtgaaacaggctcttttcaattctctgttcgtgatttcgcgtttccttcgcaattaaaatatatatcgcaaggatttttcctttccattggcatggcccttcctgccgccctaggtgttggaattgccatgcaagaccactcaaacgctcacatcaatggtggcaacgtaaaagaggactataagccaagattaattttgtttgaaggtgacggtgcagcacagatgacaatccaagaactgagcaccattctgaagtgcaatattccactagaagttatcatttggaacaataacggctacactattgaaagagccatcatgggccctaccaggtcgtataacgacgttatgtcttggaaatggaccaaactatttgaagcattcggagacttcgacggaaagtatactaatagcactctcattcaatgtccctctaaattagcactgaaattggaggagcttaagaattcaaacaaaagaagcgggatagaacttttagaagtcaaattaggcgaattggatttccccgaacagctaaagtgcatggttgaagcagcggcacttaaaagaaataaaaaatag

SEQ ID NO: 6 - DNA, 1359 bp, Synthetic construct
  source 1..1359: mol_type = other DNA
atggtatcagaggataagattgagcaatggaaagccacaaaagtcattggtataattggtctgggtgatatgggcctattatacgctaataaatttacagatgctggatggggtgttatatgttgtgatagggaagaatattatgatgaactgaaagaaaaatatgcctcagctaaattcgaactggtgaaaaatggtcatttggtatccaggcaaagcgactatattatctatagtgttgaagcatccaatattagtaagatcgtcgcaacgtatggaccatcttctaaggttggaacaattgttgggggtcaaacgagttgtaagctgccggaaatcgaggctttcgaaaagtatttacccaaggactgcgacatcattaccgtgcattcccttcatgggcctaaagttaatactgaaggccaaccactagttattatcaatcacagatcacagtacccagaatcttttgagttcgttaattctgttatggcatgtttgaaaagtaagcaagtttatttgacatatgaagagcatgacaagattaccgctgatacacaagctgtgacacatgctgctttcttaagtatgggatctgcgtgggcaaagataaagatttatccttggactctgggtgtaaacaaatggtacggtggcctagaaaatgtgaaagttaatatatcactaagaatctattcgaacaagtggcatgtttacgcaggattagccataacaaacccaagtgcacatcagcaaattcttcaatatgcaaccagtgcaacagaactatttagtttaatgatagataacaaagaacaagaacttactgatagactattaaaagctaagcaatttgtatttggaaagcatactggtctcttactattggatgacacgattttagagaaatattcgctatcaaaaagcagcattggtaacagcaacaattgcaagccagtgccgaattcacatttatcattgttggcgattgttgattcgtggtttcaacttggtattgatccatatgatcatatgatttgttcgacgccattattcagaatattcctgggtgtgtccgaatatctttttttaaaacctggcttattagaacagacaattgatgcagctatccatgataaatcattcataaaagatgatttagaatttgttatttcggctagagaatggagctcggttgtttcttttgccaattttgatatatacaaaaagcaatttcagagtgttcaaaagttctttgagccaatgcttccagaggctaatctcattggcaacgagatgataaaaaccattctgagtcattctagtgaccgttcggccgctgaaaaaagaaatacataa

SEQ ID NO: 7 - protein, 512 aa, Synthetic construct
MGSLPTNNLESISLCSQNPLDPDEFRRQGHMIIDFLADYYKNVEKYPVRSQVEPGYLKKRLPESAPYNPESIETILEDVTNDIIPGLTHWQSPNYFAYFPSSGSIAGFLGEMLSTGFNVVGFNWMSSPAATELESIVMNWLGQMLTLPKSFLFSSDGSSGGGGVLQGTTCEAILCTLTAARDKMLNKIGRENINKLVVYASDQTHCALQKAAQIAGINPKNVRAIKTSKATNFGLSPNSLQSAILADIESGLVPLFLCATVGTTSSTAVDPIGPLCAVAKLYGIWVHIDAAYAGSACICPEFRHFIDGVEDADSFSLNAHKWFFTTLDCCCLWVKDSDSLVKALSTSPEFLKNKATESKQVIDYKDWQIALSRRFRSMKLWLVLRSYGVANLRTFLRSHVKMAKHFQGLIGMDNRYEIVVPRTFAMVCFRLKPTAIFKQKIVDNDYIEDQTNEVNVKLLESVNASGKIYMTHAVVGGVYMIRFAVGATLTEERHVTGAWKVVQEHTDAILGA

SEQ ID NO: 8 - protein, 512 aa, Synthetic construct
MGSLPTNNLESISLCSQNPLDPDEFRRQGHMIIDFLADYYKNVEKYPVRSQVEPGYLKKRLPESAPYNPESIETILEDVTNDIIPGLTHWQSPNYFAYFPSSGSIAGFLGEMLSTGFNVVGFNWMSSPAATELESIVMNWLGQMLTLPKSFLFSSDGSSGGGGVLQGTTCEAILCTLTAARDKMLNKIGRENINKLVVYASDQTHCALQKAAQIAGINPKNVRAIKTSKATNFGLSPNSLQSAILADIESGLVPLFLCATVGTTSSTAVDPIGPLCAVAKLYGIWVHIDAAYAGSACICPEFRHFIDGVEDADSFSLNAHKWFFTTLDCCCLWVKDSDSLVKALSTSPEYLKNKATESKQVIDYKDWQIALSRRFRSMKLWLVLRSYGVANLRTFLRSHVKMAKHFQGLIGMDNRFEIVVPRTFAMVCFRLKPTAIFKQKIVDNDYIEDQTNEVNVKLLESVNASGKIYMTHAVVGGVYMIRFAVGATLTEERHVTGAWKVVQEHTDAILGA

SEQ ID NO: 9 - protein, 566 aa, Synthetic construct
MEFGTGNGYSNGNGYTNGNGHTNGNGNYNGNGHVNGNGKANGAKVVKMKPMDSELLREQGHIMVDFIADYYKNLQDSPQDFPVLSQVQPGYLRDMLPDSAPERPESLKELLDDVSKKIMPGITHWQSPSYFAYYASSTSVAGFLGEMLNAGLSVVGFTWLTSPAATELEIIVLDWLAKLLQLPDHFLSTGKGNGGGVIQGTGCEAVLVVVLAARDRILKKVGKTLLPQLVVYGSDQTHSSFRKACLIGGIHEENIRLLKTDSSTNYGMPPESLEEAISHDLAKGFIPFFICATVGTTSSAAVDPLVPLGNIAKKYGIWLHVDAAYAGNACICPEYRKFIDGIENADSFNMNAHKWLFANQTCSPLWVKDRYSLIDALKTNPEYLEFKVSKKDTVVNYKDWQISLSRRFRFFISPFDVVFAGPISLTNLYVHAFDLYRSLKLWMVLRLYGSENLRNFIRDHVNLAKHFEDYVAQDPSFEVVTTRYFSLVCFRLAPVDGDEDQCNERNRELLAAVNSTGKIFISHTALSGKFVLRFAVGAPLTEEKHVTEAWQIIQKHASKFTRNDHY

SEQ ID NO: 10 - protein, 472 aa, Synthetic construct
MSGTPHIAILPSPGMGHLIPMAEFAKRLVHHHNFSITFVIPTDGPPSSAYQQVLTSLPSSIDHIFLPQVDLTDVVSQSPAHPRIETLISLTVARSLSSLRTTLSSLQSSKNLVSLVVDLFGTDAFDPAIELGISPYIFFPSTAMTLSLFLYMPQLDKSVTCEFRHMTDLVRIPGCVPVRGSDLFDPVQDRTDEAYKWVIHHSNRYPMAEGVIENSFMELEHGALKYLQTVQSGKPPVYAVGPLIKMDYDVDDSGSKIIEWLDDQPVGSVLFVSFGSGGTLSYEQMTELAHGLESSQQRFLWVVRSPNQIPNSTYFSVQSQKDPLAYLPEGFLNRTEGRGLVVSNWAPQAQILSHGSTGGFMSHCGWNSILESVVHGVPIIAWPLYAEQKMNSIIVVEDVKVALRPAGVGERVVERSEITAVVKALMEGEEGKKVRNRMKELKEAAARAVSDDGASTIAIADLAQKWRSSMKH

SEQ ID NO: 11 - protein, 635 aa, Synthetic construct
MAPVTIEKFVNQEERHLVSNRSATIPFGEYIFKRLLSIDTKSVFGVPGDFNLSLLEYLYSPSVESAGLRWVGTCNELNAAYAADGYSRYSNKIGCLITTYGVGELSALNGIAGSFAENVKVLHIVGVAKSIDSRSSNFSDRNLHHLVPQLHDSNFKGPNHKVYHDMVKDRVACSVAYLEDIETACDQVDNVIRDIYKYSKPGYIFVPADFADMSVTCDNLVNVPRISQQDCIVYPSENQLSDIINKITSWIYSSKTPAILGDVLTDRYGVSNFLNKLICKTGIWNFSTVMGKSVIDESNPTYMGQYNGKEGLKQVYEHFELCDLVLHFGVDINEINNGHYTFTYKPNAKIIQFHPNYIRLVDTRQGNEQMFKGINFAPILKELYKRIDVSKLSLQYDSNVTQYTNETMRLEDPTNGQSSIITQVHLQKTMPKFLNPGDVVVCETGSFQFSVRDFAFPSQLKYISQGFFLSIGMALPAALGVGIAMQDHSNAHINGGNVKEDYKPRLILFEGDGAAQMTIQELSTILKCNIPLEVIIWNNNGYTIERAIMGPTRSYNDVMSWKWTKLFEAFGDFDGKYTNSTLIQCPSKLALKLEELKNSNKRSGIELLEVKLGELDFPEQLKCMVEAAALKRNKK

SEQ ID NO: 12 - protein, 452 aa, Synthetic construct
MVSEDKIEQWKATKVIGIIGLGDMGLLYANKFTDAGWGVICCDREEYYDELKEKYASAKFELVKNGHLVSRQSDYIIYSVEASNISKIVATYGPSSKVGTIVGGQTSCKLPEIEAFEKYLPKDCDIITVHSLHGPKVNTEGQPLVIINHRSQYPESFEFVNSVMACLKSKQVYLTYEEHDKITADTQAVTHAAFLSMGSAWAKIKIYPWTLGVNKWYGGLENVKVNISLRIYSNKWHVYAGLAITNPSAHQQILQYATSATELFSLMIDNKEQELTDRLLKAKQFVFGKHTGLLLLDDTILEKYSLSKSSIGNSNNCKPVPNSHLSLLAIVDSWFQLGIDPYDHMICSTPLFRIFLGVSEYLFLKPGLLEQTIDAAIHDKSFIKDDLEFVISAREWSSVVSFANFDIYKKQFQSVQKFFEPMLPEANLIGNEMIKTILSHSSDRSAAEKRNT

SEQ ID NO: 13 - DNA, 55 bp, Synthetic construct
  source 1..55: mol_type = other DNA
ttaacgtcaaggagaaaaaaccccggatccatggtatcagaggataagattgagc

SEQ ID NO: 14 - DNA, 55 bp, Synthetic construct
  source 1..55: mol_type = other DNA
tagctagccgcggtaccaagcttactcgagttatgtatttcttttttcagcggcc

SEQ ID NO: 15 - DNA, 60 bp, Synthetic construct
  source 1..60: mol_type = other DNA
tccttgtaatccatcgatactagtgcggccgcctattttttatttcttttaagtgccgct

SEQ ID NO: 16 - DNA, 55 bp, Synthetic construct
  source 1..55: mol_type = other DNA
tcgaattcaaccctcactaaagggcggccgcatggcacctgttacaattgaaaag

SEQ ID NO: 17 - DNA, 59 bp, Synthetic construct
  source 1..59: mol_type = other DNA
ttgtacaactgtgctaaacagacttaaaaaagtaataattgagcgacctcatgctatac

SEQ ID NO: 18 - DNA, 59 bp, Synthetic construct
  source 1..59: mol_type = other DNA
ctattggagtgatcaaaaaaaacttcaattagcgtgataccttcgagcgtcccaaaacc

SEQ ID NO: 19 - DNA, 59 bp, Synthetic construct
  source 1..59: mol_type = other DNA
acactcgcgagaaccaaaacaaggatcccctaaacccagtatccgctctaaccgaaaag

SEQ ID NO: 20 - DNA, 59 bp, Synthetic construct
  source 1..59: mol_type = other DNA
aagcgatccgtagtcctatccgggtaacactcatcgtccgcttcgagcgtcccaaaacc

SEQ ID NO: 21 - DNA, 59 bp, Synthetic construct
  source 1..59: mol_type = other DNA
tcgtgttcatgcagatagataacaatctatatgttgataagagcgacctcatgctatac

SEQ ID NO: 22 - DNA, 59 bp, Synthetic construct
  source 1..59: mol_type = other DNA
cataaaagaccgtgtgatggcttggcatggcgatttcattcttcgagcgtcccaaaacc

SEQ ID NO: 23 - DNA, 24 bp, Synthetic construct
  source 1..24: mol_type = other DNA
aaagctacatataaggaacgtgct

SEQ ID NO: 24 - DNA, 22 bp, Synthetic construct
  source 1..22: mol_type = other DNA
caggctgggaagcatatttgag

SEQ ID NO: 25 - DNA, 24 bp, Synthetic construct
  source 1..24: mol_type = other DNA
ttcatttaccggcgcactctcgcc

SEQ ID NO: 26 - DNA, 23 bp, Synthetic construct
  source 1..23: mol_type = other DNA
taaataagaacacccgcatgcac

SEQ ID NO: 27 - DNA, 23 bp, Synthetic construct
  source 1..23: mol_type = other DNA
agagcagaaagccctagtaaagc

SEQ ID NO: 28 - DNA, 22 bp, Synthetic construct
  source 1..22: mol_type = other DNA
aacatcgttggtaccattgggc